European Patent Specification EP 3 662 068 B1, published October 18, 2023. Title: FUNGAL CELL WITH IMPROVED PROTEIN PRODUCTION CAPACITY. Applicant: Biopetrolia AB. The sequence listing filed with the application follows.

SEQUENCE LISTING (77 sequences)

SEQ ID NO: 1 - protein, 523 aa, Saccharomyces cerevisiae
MGEDFMHPPFQTYPSKNSEGKKHIVIVGGGIIGCCTAYYLTQHPSFSPSTHHITIIESRRIAGGASGKAGGLLASWAFPHQIVPLSFQLHQELSDEYDGENNWDYRRLTTVSLEADVREEVIENYERLSKKAYNLNVPPPKKRPGYISNKFNIGDSNSSLSSSGSSLKNDSASNEEEGSDIHVSSSVPSLHSLTNERMRSHTNSASDLDSVSPVEQLRETNIHNPLPADLDWIRRELVNDWSSLGGTDTTAQLHPYKFTHFILSKAMETGAVDLLLGKVVGLKCDEMDCVHSLKYLPSVVKNRRNSRGHAENPDIKLGTIFNDENAKPIEINDIQQIVLSMGPWTSKILKDCPISGLRAHSVTIKPSEKTVSPYAILAELKVNDREFFSPEMYARKDEVYVCGEGDTLVNIPESSDDVEVVSEKCDELYHYVSKLSPTLSKGHLLRKQACFLPVLNVPTSSGPLIGETNVKDLYIASGHSCWGINNAPATGKLMAEILLDGEATSAEISSLDPKLYFDATILS

SEQ ID NO: 2 - protein, 223 aa, Saccharomyces cerevisiae
MSSQPSFVTIRGKAISLETQTESLLSKYSTFAQTTSSEQTGQEKKIDKQLEGILGQRQDVIDSLTQICDSNPAISASKLSQLHRHKEILQDHWKSFRNIRSSIQQERNRLNLLFSVKNDIANSTTDAPAPIGDADEYIQNETRRIDQSNNVVDRLISQAWETRSQFHSQSNVLNTANNKVLQTLQRIPGVNQLIMKINTRRKKNAFVLATITTLCILFLFFTW

SEQ ID NO: 3 - protein, 675 aa, Saccharomyces cerevisiae
MDYEDNLEAPVWDELNHEGDKTQSLVSNSIESIGQISTNEERKDNELLETTASFADKIDLDSAPEWKDPGLSVAGNPQLEEHDNSKADDLINSLAPEQDPIADLKNSTTQFIATRESGGALFTGNANSPLVFDDTIYDANTSPNTSKSISGRRSGKPRILFDSARAQRNSKRNHSLKAKRTTASDDTIKTPFTDPLKKAEKENEFVEEPLDDRNERRENNEGKFTASVEKNILEQVDRPLYNLPQTGANISSPAEVEENSEKFGKTKIGSKVPPTEKAVAFKVEVKDPVKVGELTSIHVEYTVISESSLLELKYAQVSRRYRDFRWLYRQLQNNHWGKVIPPPPEKQSVGSFKENFIENRRFQMESMLKKICQDPVLQKDKDFLLFLTSDDFSSESKKRAFLTGSGAINDSNDLSEVRISEIQLLGAEDAAEVLKNGGIDAESHKGFMSISFSSLPKYNEADEFFIEKKQKIDELEDNLKKLSKSLEMVDTSRNTLAASTEEFSSMVETLASLNVSEPNSELLNNFADVHKSIKSSLERSSLQETLTMGVMLDDYIRSLASVKAIFNQRSKLGYFLVVIENDMNKKHSQLGKLGQNIHSEKFREMRKEFQTLERRYNLTKKQWQAVGDKIKDEFQGFSTDKIREFRNGMEISLEAAIESQKECIELWETFYQTNL

SEQ ID NO: 4 - protein, 551 aa, Saccharomyces cerevisiae
MTSAVPYDPYDDLDNNPFAEPQEEDSEPAATTTDGSSSMSEERVGTEQTAASVQDNGTANNIQNGLGEEGNATRSKTSNEHNENQQPSQPSERVILPERSDEKKKYTLLAKVTGLERFGSATGKKENPTIIFDCSTNLPTFRKQQYKNVKKSYEEFHQLFKYLNVAIQESFVPTLPSAYTTFGINSEEDRMKVTRNFQLWFNRLSQDPLIIRNEEVAFFIESDFNTYTPINKSKSLASGLKRKTLKQLAPPYDEITELAEFRPLVKSIYVVSQSLQEKLLRVSRNRKMMVQEENAFGQDFVNLDEHNKLYRRYGKILTAVGDIDSIIATMDMATLYDGLEWIVRDAYAVKEALTNRHFIMRNLVQAQQNSKAKQEQARRFRSRRDINPMKIDEALRQLKAAAKNEQVLTLKLQRITSNMIIERKQWISWYEEWIRSSIKEFTLRKIEYERKKLTLLERVRSDIRKADENGGLSRLGRHAVSNNNSDTSQTLKGDSWTGESNRKSQIPINKIAHTEFDDELFTEDDGYNSQDSDTTSLNARHAASLLGMSTK

SEQ ID NO: 5 - protein, 379 aa, Saccharomyces cerevisiae
MSIFFKPPIDIEILFDNEESRKHVDIATRSSNSSYKSMKESLPVYEDGESLGGIVTLRVRDSKKVDHLGIKVSVIGSIDMLKSHGSGNSSSKKVTSSTSSSSSNGSVDVRKNSVDQFLCQSYDLCPAGELQHSQSFPFLFRDLSKRYESYKGKNVDVAYYVKVTVMRKSTDISKIKRFWVYLYNSVTTAPNTLSANETKATTNDIAGGNYAADNASDNTQTKSTQGEAADVNQVLPISHSNNEPKPVRLDIGIENCLHIEFEYAKSQYSLKEVIVGRIYFLLTRLRIKHMELSLITRESSGLQTSNVMTDSTAIRYEIMDGSSVKGETIPIRLFLSGYDLTPNMSCNYFNVKNYLSLVIIDEDGRRYFKQSEITLYRTR

SEQ ID NO: 6 - protein, 282 aa, Saccharomyces cerevisiae
MLLLALSDAHIPDRATDLPVKFKKLLSVPDKISQVALLGNSTKSYDFLKFVNQISNNITIVRGEFDNGHLPSTKKDKASDNSRPMEEIPMNSIIRQGALKIGCCSGYTVVPKNDPLSLLALARQLDVDILLWGGTHNVEAYTLEGKFFVNPGSCTGAFNTDWPIVFDVEDSDEAVTSEVDKPTKENQSEDDDAKGGSTGKEQPGSYTPKEGTAGERENENESNVKPENQFKEDEVDMSDSDINGSNSPSFCLLDIQGNTCTLYIYLYVNGEVKVDKVVYEKE

SEQ ID NO: 7 - protein, 944 aa, Saccharomyces cerevisiae
MAYADSPENAIAVIKQRTALMNRCLSQHKLMESLQHTSIMLTELRNPNLSPKKYYELYVIIFDSLTNLSTYLIENHPQNHHLADLYELVQYTGNVVPRLYLMITVGTSYLTFNEAPKKEILKDMIEMCRGVQNPIRGLFLRYYLSQRTKELLPEDDPSFNSQFIMNNFIEMNKLWVRLQHQGPLRERETRTRERKELQILVGSQLVRLSQIIDDNFQMYKQDILPTILEQVIQCRDLVSQEYLLDVICQVFADEFHLKTLDTLLQTTLHLNPDVSINKIVLTLVDRLNDYVTRQLEDDPNATSTNAYLDMDVFGTFWDYLTVLNHERPDLSLQQFIPLVESVIVLSLKWYPNNFDNLNKLFELVLQKTKDYGQKNISLESEHLFLVLLSFQNSKLQLTSSTTAPPNSPVTSKKHFIFQLISQCQAYKNILALQSISLQKKVVNEIIDILMDREVEEMADNDSESKLHPPGHSAYLVIEDKLQVQRLLSICEPLIISRSGPPANVASSDTNVDEVFFNRHDEEESWILDPIQEKLAHLIHWIMNTTSRKQTMKNKIQFSLEAQLEILLLIKSSFIKGGINVKYTFPAIITNFWKLMRKCRMIQEYLLKKRPDNKTLLSHYSNLLKQMFKFVSRCINDIFNSCNNSCTDLILKLNLQCAILADQLQLNEISYDFFSQAFTIFEESLSDSKTQLQALIYIAQSLQKTRSLYKEAYYDSLIVRCTLHGSKLLKKQDQCRAVYLCSHLWWATEISNIGEEEGITDNFYRDGKRVLECLQRSLRVADSIMDNEQSCELMVEILNRCLYYFIHGDESETHISIKYINGLIELIKTNLKSLKLEDNSASMITNSISDLHITGENNVKASSNADDGSVITDKESNVAIGSDGTYIQLNTLNGSSTLIRGVVATASGSKLLHQLKYIPIHHFRRTCEYIESQREVDDRFKVIYV

SEQ ID NO: 8 - protein, 674 aa, Saccharomyces cerevisiae
MSRKNSKKLKVYYLPVTLTQFQKDLSEILISLHAKSFKASLIGEPQADAVNKPSGLPAGPETHPYPTLSQRQLTYIFDSNIRAIANHPSLLVDHYMPRQLLRMEPTESSIAGSHKFQVLNQLINSICFRDREGSPNEVIKCAIIAHSIKELDLLEGLILGKKFRTKRLSGTSLYNEKHKFPNLPTVDSTINKDGTPNSVSSTSSNSNSTSYTGYSKDDYDYSVKRNLKKRKINTDDWLFLATTKHLKHDQYLLANYDIDMIISFDPMLEIELPALQVLRNNANKDIPIIKLLVQNSPDHYLLDSEIKNSSVKSSHLSNNGHVDDSQEYEEIKSSLLYFLQARNAPVNNCEIDYIKLVKCCLEGKDCNNILPVLDLITLDEASKDSSDSGFWQPQLTKLQYSSTELPLWDGPLDIKTYQTDLMHRAVIRLRDIQDEYAKGTVPLYEKRLNETQRQNQLDEIKNSVGLTFKKKQEMEKSINDSEKRLKHAMTESTKLQNKINHLLKIRQELENFNKLPSNTTSSENHLEEGSALADKLKEYIDKNATLFNKLKELQQANAEKSKLNDELRSKYQIESSKAAESAQTLKILRESMKSLENEVNGPLTKFSTESLKKELERLQNDFQSLKARNKFLKNYITLMNRQYDLKNKNNVQVEKAAANGTRFRSTRSNTPNYT

SEQ ID NO: 9 - protein, 655 aa, Saccharomyces cerevisiae
MDLLRILDTKPIPTIVDATTLGISGNTSGDYWLPTTMSLYQKELTDQIVSLHYSDILRYFETSHYKEDVILESMKTMCLNGSLVATHPYLLIDHYMPKSLITRDVPAHLAENSGKFSVLRDLINLVQEYETETAIVCRPGRTMDLLEALLLGNKVHIKRYDGHSIKSKQKANDFSCTVHLFSSEGINFTKYPIKSKARFDMLICLDTTVDTSQKDIQYLLQYKRERKGLERYAPIVRLVAINSIDHCTLFFGKKFDKNSREYLENVTAAMVILRDRLGTLPPDLRPIYSQKLHYLVEWLENPTVPWPLPDIYPLKQYTSMDVERSLLTEVHFKKSDDQLEDAFSNCSKKRGRHGANKAASSTVAGIEDNITPSFYSTKRLKNDYYTNPLKQDMTQLTGITTADNSSNVNYHLSSGIITHKLIQSMGEVYMDICVQKQELDDYSCLDDLQNDHLKFFSNEDEKIIKEYETVLRTNNDNLNRSHELEVENNLKFSQIETLEKDIETLKGSLMAQGETLSKLKDAFVKTDNVQDEIEKEERISVSRDTEKKYMEQEIKRAVDAIRENEEETHKLNEKKNGLESELKLKFGKSEISTKELNEKIGFLKKELKLENDLNEELMGQLSKTMDNLENLTIPRVRTQNGNTKKKSKAKKPGNV

SEQ ID NO: 10 - protein, 569 aa, Saccharomyces cerevisiae
MSFQIETVPTKPYEDQKPGTSGLRKKTKVFKDEPNYTENFIQSIMEAIPEGSKGATLVVGGDGRYYNDVILHKIAAIGAANGIKKLVIGQHGLLSTPAASHIMRTYEEKCTGGIILTASHNPGGPENDMGIKYNLSNGGPAPESVTNAIWEISKKLTSYKIIKDFPELDLGTIGKNKKYGPLLVDIIDITKDYVTFLKEIFDFDLIKKFIDNQRSTKNWKLLFDSMNGVTGPYGKAIFVDEFGLPADEVLQNWHPSPDFGGMHPDPNLTYASSLVKRVDREKIEFGAASDGDGDRNMIYGYGPSFVSPGDSVAIIAEYAAEIPYFAKQGIYGLARSFPTSGAIDRVAKAHGLNCYEVPTGWKFFCALFDAKKLSICGEESFGTGSNHVREKDGVWAIMAWLNILAIYNKHHPENEASIKTIQNEFWAKYGRTFFTRYDFEKVETEKANKIVDQLRAYVTKSGVVNSAFPADESLKVTDCGDFSYTDLDGSVSDHQGLYVKLSNGARFVLRLSGTGSSGATIRLYIEKYCDDKSQYQKTAEEYLKPIINSVIKFLNFKQVLGTEEPTVRT

SEQ ID NO: 11 - protein, 870 aa, Saccharomyces cerevisiae
MSTTLAAPAKLKSLLLNLHTHCIGLHVNDVTPKVYFKLLIRHLLQISRSNAAHPKLRRRAQILLVSLFLSGVTLFSGVTYSTFKIILKCYKFYKFPWKRRNRRPLIRRTRSQMQLDSGARIMYIPEVELVDRQSPDDNKFMNATDKKKRKRIFIPPKDNDVYEHDKFLFKNVELERAKNSQLFYSKFLNQMNVLSKILIPTVFDKNFLLLTAQIFFLVMRTWLSLFVAKLDGQIVKNIIAGRGRSFLWDLGCWFLIAVPASYTNSAIKLLQRKLSLNFRVNLTRYIHDMYLDKRLTFYKLIFDAKASNSVIKNIDNSITNDVAKFCDATCSVFANIAKPVIDLIFFSVYLRDNLGTVGVAGIFVNYFITGFILRKYTPPLGKLAGERSASDGDYYNYHLNMINNSEEIAFYQGTAVERTKVKELYDVLMEKMLLVDKVKFGYNMLEDYVLKYTWSGLGYVFASIPIVMSTLATGINSEEKNMKEFIVNKRLMLSLADAGSRLMHSIKDISQLTGYTNRIFTLLSVLHRVHSLNFNYGAVPSILSIRTEDASRNSNLLPTTDNSQDAIRGTIQRNFNGIRLENIDVIIPSVRASEGIKLINKLTFQIPLHIDPITSKSNSIQDLSKANDIKLPFLQGSGSSLLILGPNGCGKSSIQRIIAEIWPVYNKNGLLSIPSENNIFFIPQKPYFSRGGTLRDQIIYPMSSDEFFDRGFRDKELVQILVEVKLDYLLKRGVGLTYLDAIADWKDLLSGGEKQRVNFARIMFHKPLYVVLDEATNAISVDMEDYLFNLLKRYRFNFISISQRPTLIKYHEMLLEIGENRDGKWQLQAVGTDEAITSIDNEIEELERKLERVKGWEDERTKLREKLEII

SEQ ID NO: 12 - protein, 853 aa, Saccharomyces cerevisiae
MISTASAFYQKHRVNLLRSSYIILLLATLYNSNSSSSNNKTDKKDSESTVLENKKIEEGKETAVDREEDESSKEELTIVSKHSTDSEDGAIIIDKESKTNHKGGERKGKVDFLFKLLLHDKKCLILFITQAILLNIRTLLSLRVATLDGQLVSTLVRAQYANFTKILLGKWMILGIPASFINSLISYTTKLCAVTINRKVSDFLLSKYLSNHHTFYSVASAESVSEIQDNLTKDIYTFSMNSSLLLNQLLKPMLDLILCSFKLLTSNTSVMGEGTLALGLIVYASNSLLKLIQPNFTRLTMASASLESWFRSLHSNLHSSNEEIALLRGQKRELENVDYSFYRLVLFLNREIKARAIYDVATAFVIKYTWGAAGLVLCSIPIFFKNKPSEDTLQLKEPGNDMTADFITNRRLLVTASSSIGRFVELKRNIQQLRGIRLRLNKFNDLLDANKGDDEKEPRDERCIVEYDDSRIKFENIPLITPANQVLVPELSFDLKHGNHLLIIGPNGCGKSSLFRILGGLWPIRATPNKNHQSKLIMPRRTVDRDCAIFYLPQRPYMGNRSTFREQIIYPDSIEQFKERYHNDYDLGDADLIKILQLLDLEDLVTENMSLLLAQRTSKNDSQQLSTEDNQSPCAIKVRDAFSIVRNWSEELTIGVQQRLAMARMYYHKPKFAVLDECTSAVAPEMEQRMYENAQNFGISLISVCHRTSLWHFHNYLLKFDGKGGYQFGPFNPKERLCNEEKLLELNAILDQQVPLWERKLKDLTIAKESNIIRKSETNLNLFEKIEDPKTSKSNALFNANKGQRITSPTGQETSKRLPLFSQPSSSASSNLLRNNKSLNKKVKTKKEEGKER

SEQ ID NO: 13 - protein, 760 aa, Saccharomyces cerevisiae
MKITCTDLVYVFILLFLNTSCVQAVFSDDAFITDWQLANLGPWEKVIPDSRDRNRVLILSNPTETSCLVSSFNVSSGQILFRNVLPFTIDEIQLDSNDHNAMVCVNSSSNHWQKFDLHDWFLLEEGVDNAPSTTILPQSSYLNDQVSIKNNELHILDEQSKLAEWKLELPQGFNKVEYFHREDPLALVLNVNDTQYMGFSANGTELIPVWQRDEWLTNVVDYAVLDVFDSRDVELNKDMKAELDSNSLWNAYWLRLTTNWNRLINLLKENQFSPGRVFTKLLALDAKDTTVSDLKFGFAKILIVLTHDGFIGGLDMVNKGQLIWKLDLEIDQGVKMFWTDKNHDELVVFSHDGHYLTIEVTKDQPIIKSRSPLSERKTVDSVIRLNEHDHQYLIKFEDKDHLLFKLNPGKNTDVPIVANNHSSSHIFVTEHDTNGIYGYIIENDTVKQTWKKAVNSKEKMVAYSKRETTNLNTLGITLGDKSVLYKYLYPNLAAYLIANEEHHTITFNLIDTITGEILITQEHKDSPDFRFPMDIVFGEYWVVYSYFSSEPVPEQKLVVVELYESLTPDERLSNSSDNFSYDPLTGHINKPQFQTKQFIFPEIIKTMSISKTTDDITTKAIVMELENGQITYIPKLLLNARGKPAEEMAKDKKKEFMATPYTPVIPINDNFIITHFRNLLPGSDSQLISIPTNLESTSIICDLGLDVFCTRITPSGQFDLMSPTFEKGKLLITIFVLLVITYFIRPSVSNKKLKSQWLIK

SEQ ID NO: 14 - protein, 117 aa, Saccharomyces cerevisiae
MSSSTPFDPYALSEHDEERPQNVQSKSRTAELQAEIDDTVGIMRDNINKVAERGERLTSIEDKADNLAVSAQGFKRGANRVRKAMWYKDLKMKMCLALVIIILLVVIIVPIAVHFSR

SEQ ID NO: 15 - protein, 115 aa, Saccharomyces cerevisiae
MSSSVPYDPYVPPEESNSGANPNSQNKTAALRQEIDDTVGIMRDNINKVAERGERLTSIEDKADNLAISAQGFKRGANRVRKQMWWKDLKMRMCLFLVVIILLVVIIVPIVVHFS

SEQ ID NO: 16 - protein, 403 aa, Saccharomyces cerevisiae
MTIAPMANDLEDFESLLEPTFDAKQFGNDLLKATNNNDTTILDLNTPLKKLNYDLHEIDSRIDQLMNSNPLEIIELIYKNEHVNSTIVGELKPSLEYMNMSYDRLKNQVLDPYERARKVQLALSKVYQTSFLLRGALLYIHLSNKLNALSKTAQLSTSTAINLASLHYQLEITLDENKNLKSLRKIKQLDQDIVSPNKRELITFLSLQMCKECLNSIKIKSNKEIISQLAYSLYLLSSQEFESAINKIVLSNVTMSSQILSKILNSIRMFPDAFNEVVEKGYNIYILETLLRNIKTDNVTNSSRSIAANKSRLGNLLSEYTSMKSKAGSGTPRDLFWSKVSSAFKKDFEISVNRGGPVGKSLLKNKDFIINTMKQSMKKSSDNSDYQSYLDVMLNSVSISLNK

SEQ ID NO: 17 - DNA, 1569 bp, Saccharomyces cerevisiae
atgaagttttctgctggtgccgtcctgtcatggtcctccctgctgctcgcctcctctgttttcgcccaacaagaggctgtggcccctgaagactccgctgtcgttaagttggccaccgactccttcaatgagtacattcagtcgcacgacttggtgcttgcggagttttttgctccatggtgtggccactgtaagaacatggctcctgaatacgttaaagccgccgagactttagttgagaaaaacattaccttggcccagatcgactgtactgaaaaccaggatctgtgtatggaacacaacattccagggttcccaagcttgaagattttcaaaaacagcgatgttaacaactcgatcgattacgagggacctagaactgccgaggccattgtccaattcatgatcaagcaaagccaaccggctgtcgccgttgttgctgatctaccagcttaccttgctaacgagacttttgtcactccagttatcgtccaatccggtaagattgacgccgacttcaacgccaccttttactccatggccaacaaacacttcaacgactacgactttgtctccgctgaaaacgcagacgatgatttcaagctttctatttacttgccctccgccatggacgagcctgtagtatacaacggtaagaaagccgatatcgctgacgctgatgtttttgaaaaatggttgcaagtggaagccttgccctactttggtgaaatcgacggttccgttttcgcccaatacgtcgaaagcggtttgcctttgggttacttattctacaatgacgaggaagaattggaagaatacaagcctctctttaccgagttggccaaaaagaacagaggtctaatgaactttgttagcatcgatgccagaaaattcggcagacacgccggcaacttgaacatgaaggaacaattccctctatttgccatccacgacatgactgaagacttgaagtacggtttgcctcaactctctgaagaggcgtttgacgaattgagcgacaagatcgtgttggagtctaaggctattgaatctttggttaaggacttcttgaaaggtgatgcctccccaatcgtgaagtcccaagagatcttcgagaaccaagattcctctgtcttccaattggtcggtaagaaccatgacgaaatcgtcaacgacccaaagaaggacgttcttgttttgtactatgccccatggtgtggtcactgtaagagattggccccaacttaccaagaactagctgatacctacgccaacgccacatccgacgttttgattgctaaactagaccacactgaaaacgatgtcagaggcgtcgtaattgaaggttacccaacaatcgtcttatacccaggtggtaagaagtccgaatctgttgtgtaccaaggttcaagatccttggactctttattcgacttcatcaaggaaaacggtcacttcgacgtcgacggtaaggccttgtacgaagaagcccaggaaaaagctgctgaggaagccgatgctgacgctgaattggctgacgaagaagatgccattcacgatgaattgtaa

SEQ ID NO: 18 - DNA, 2502 bp, Saccharomyces cerevisiae
atgaataatgctgcaaatacagggacgaccaatgagtcaaacgtgagcgatgctccccgtattgagcctttaccaagcttgaatgatgatgacattgaaaaaatcttacaaccgaacgatatctttacgaccgatcgtaccgatgcaagtactacatcttccacagccattgaagatattattaacccctcattggatccgcagtcagcagcatcgccggttccttcttcctcttttttccatgactcaaggaaaccttccaccagtacacatttagtaaggagaggtactccattgggaatttaccaaaccaatctatacggtcacaatagcagagaaaatactaatcctaatagtacattattatcttctaagttactcgcgcatccaccagttccttatgggcaaaatcccgatttactacaacatgctgtgtacagggcacagccgtcaagtggaaccactaacgcgcaaccgcgccaaaccacaagaagatatcaatcccataaatcacggcctgcatttgttaataaactatggagcatgttaaacgatgattctaatacgaaacttatacagtgggcggaggatggaaaatcttttattgtcacgaatagggaggaatttgtgcaccaaattttaccaaaatattttaaacattccaatttcgcttcctttgtaagacaattgaacatgtatggatggcataaagttcaagatgtcaagtcaggatcaattcaaagtagttcagatgataagtggcaatttgaaaatgaaaacttcattagaggtagagaagatttgctggaaaaaataatcaggcagaaaggttcctccaataaccataatagccctagtggtaacggtaatccagcgaatggtagcaacatccctctggacaatgccgcaggaagtaataatagcaataataacatcagtagtagtaattcattttttaacaatggtcatttattgcagggtaaaacactaagattaatgaacgaagcgaatcttggagataagaatgatgtcaccgcgattttgggggaattagagcaaataaaatataaccagattgcaatttccaaagatttactaagaataaacaaagataatgagttattatggcaagagaatatgatggccagggaaagacatagaacccaacagcaagccttggaaaaaatgttcagattcttgacatctatagtcccacacttagatcccaaaatgattatggacgggctgggagatccgaaagttaataatgaaaagctaaacagtgcgaataacattgggttaaatcgcgacaacacaggcactatagatgaactaaaatccaacgattctttcataaacgatgatcgtaattctttcaccaatgctacaaccaacgcccgtaataacatgagtcccaacaatgatgacaatagtattgacaccgctagcactaataccaccaacagaaagaaaaatatagatgaaaacatcaaaaataacaacgacataattaatgacattatatttaataccaaccttgccaacaatctcagcaattacaattccaacaataatgctggctcgccaataaggccctataaacaaagatatcttttgaaaaatagagccaattcctcgacatcgagtgagaatccaagcctaacgccctttgatatcgaatctaataatgaccgcaaaatttcagaaattccttttgatgacgaagaagaagaagaaacggattttaggccttttacctcgcgagatcctaataaccaaacgagtgaaaacacttttgatccaaacagatttacgatgctctctgatgatgatttaaaaaaagattctcataccaatgacaataaacacaacgaaagtgatcttttttgggacaacgtacatagaaatatagacgaacaagatgcaagactccagaacttggaaaatatggttcacatactttctcctggatatcctaataagtcgttcaacaacaaaacttcctcgacaaacactaattccaatatggaaagtgctgtcaacgttaatagccctggtttcaacttacaggattatttaactggagagtctaattcccccaattctgttcattctgttccctccaatggcagcggctccacaccgttgcccatgccaaatgataatgacaccgagcacgcaagtacaagtgtcaatcaaggcgaaaatggaagcggattaacgcccttcctcacggtagatgatcacacactaaacgacaataacactagtgagggaagtacaagggtgtcccccgatataaagttcagcgccactgaaaacactaaagtgagtgataacctgccaagctttaatgaccacagttattccacccaggccgacacggcgcccgagaacgctaagaaaagatttgtggaggaaataccggaaccggctatagtcgaaatacaggacccgacagagtacaacgatcaccgcctgcccaaacgagctaagaaatag

SEQ ID NO: 19 - protein, 238 aa, Saccharomyces cerevisiae
MEMTDFELTSNSQSNLAIPTNFKSTLPPRKRAKTKEEKEQRRIERILRNRRAAHQSREKKRLHLQYLERKCSLLENLLNSVNLEKLADHEDALTCSHDAFVASLDEYRDFQSTRGASLDTRASSHSSSDTFTPSPLNCTMEPATLSPKSMRDSASDQETSWELQMFKTENVPESTTLPAVDNNNLFDAVASPLADPLCDDIAGNSLPFDNSIDLDNWRNPEAQSGLNSFELNDFFITS

SEQ ID NO: 20 - DNA, 41 bp, Primer
actgcggccgcaacaaaatgtcttacagaggacctattgga

SEQ ID NO: 21 - DNA, 40 bp, Primer
cgtgagctcctagtaaatcttcttcttttcatcaacggat

SEQ ID NO: 22 - DNA, 37 bp, Primer
tcaggatccaacaaaatgacaatagcgccaatggcaa

SEQ ID NO: 23 - DNA, 45 bp, Primer
ccaggtacctcacttatttagagaaatagatactgagtttagcat

SEQ ID NO: 24 - DNA, 38 bp, Primer
actgcggccgcaacaaaatgaagttttctgctggtgcc

SEQ ID NO: 25 - DNA, 37 bp, Primer
cgtgagctcttacaattcatcgtgaatggcatcttct

SEQ ID NO: 26 - DNA, 80 bp, Primer
atgagtaggaaaaattctaagaaactaaaagtctattacttacctgtaacgctaacccaagacatggaggcccagaatac

SEQ ID NO: 27 - DNA, 113 bp, Primer
aaatctctctatattatacaggctacttcttttaggaaacgtcacattcattagtcgatagtattgtatctattttctttatttttcacacaccagtatagcgaccagcattc

SEQ ID NO: 28 - DNA, 83 bp, Primer
atggactacgaggataatctagaagcacctgtttgggacgaactaaatcatgagggagataaagacatggaggcccagaatac

SEQ ID NO: 29 - DNA, 113 bp, Primer
ataaatcctgaggaacgtgacacataaagttattgtatacagatcatctattaggcttgttattgcaggatgtatgaaagtttataaaatccccagtatagcgaccagcattc

SEQ ID NO: 30 - DNA, 84 bp, Primer
atgagctcacaaccgtctttcgtcaccataaggggcaaggccatttctctagaaacacaaacgggacatggaggcccagaatac

SEQ ID NO: 31 - DNA, 113 bp, Primer
agattcttgttatgtttttacatacgttgtttaataaaagtcgttatttatcagtggtgtggttgcttgtctggaattgggcttttccctgtgcagtatagcgaccagcattc

SEQ ID NO: 32 - DNA, 82 bp, Primer
atgggtgaagattttatgcacccaccgtttcaaacgtacccttcaaagaacagcgaagggaagacatggaggcccagaatac

SEQ ID NO: 33 - DNA, 113 bp, Primer
caaatttgtgcatatacttttcttgaccttattactcctcggcttgattatcattataaacactattccttctgttgcttggttaaaatgctacagtatagcgaccagcattc

SEQ ID NO: 34 - DNA, 92 bp, Primer
atgacttcggctgtaccttatgatccatatgatgatctggataacaatccatttgctgagccccaggaggaagacatggaggcccagaatac

SEQ ID NO: 35 - DNA, 117 bp, Primer
aaagatcaccttgttcaaaggtatgaattttctactttatatacgtattatcatgttcagaggatagatggattgactaagggtacagtacggcaaacagtatagcgaccagcattc

SEQ ID NO: 36 - DNA, 20 bp, Primer
gacatggaggcccagaatac

SEQ ID NO: 37 - DNA, 20 bp, Primer
cagtatagcgaccagcattc

SEQ ID NO: 38 - DNA, 117 bp, Primer
ttctagaagatgagagaagagggaataatgagaaaggcgaaaaataaaggcacacaccatagcttcaaaatgtttctactccttttttactcttccagacatggaggcccagaatac

SEQ ID NO: 39 - DNA, 87 bp, Primer
aagttaagtgcgcagaaagtaatatcatgcgtcaatcgtatgtgaatgctggtcgctatactggcacacaccatagcttcaaaatgt

SEQ ID NO: 40 - DNA, 24 bp, Primer
gacaaacttggaatgtaaggcttc

SEQ ID NO: 41 - DNA, 118 bp, Primer
attttttgttagacatataattttatatcattattcttattattcttataggaagtaccttcaaagaatggggtcttatcttgttttgcaagtaccacgacatggaggcccagaatac

SEQ ID NO: 42 - DNA, 88 bp, Primer
aagttaagtgcgcagaaagtaatatcatgcgtcaatcgtatgtgaatgctggtcgctatactgggaagtaccttcaaagaatggggtc

SEQ ID NO: 43 - DNA, 25 bp, Primer
tatctccaatgggttgctattcatc

SEQ ID NO: 44 - DNA, 118 bp, Primer
gcattttgttgtgctgttacaaccacaacaaaacgaaaaacccgtatggatccaactggcaccgctggcttgaacaacaataccagccttccaacttcgacatggaggcccagaatac

SEQ ID NO: 45 - DNA, 84 bp, Primer
aagttaagtgcgcagaaagtaatatcatgcgtcaatcgtatgtgaatgctggtcgctatactgtccaactggcaccgctggctt

SEQ ID NO: 46 - DNA, 117 bp, Primer
acagcctcttgttgggcgaaaacagaggaggcgagcagcagggaggaccatgacaggacggcaccagcagaaaacttcattttgaatatgtattacttggttatggttatatatgac

SEQ ID NO: 47 - DNA, 118 bp, Primer
gttcaatagtgtggttggtaaccaaattttctaggcgttgttgaaaataatcattagtgcccaccgtttgagcgtggtgtgacaccacgcccaagatagacatggaggcccagaatac

SEQ ID NO: 48 - DNA, 95 bp, Primer
cccagatgcgaagttaagtgcgcagaaagtaatatcatgcgtcaatcgtatgtgaatgctggtcgctatactgtcattagtgcccaccgtttgag

SEQ ID NO: 49 - DNA, 99 bp, Primer
attacgaaatggcctgtatgggtagattcttgttatgtttttacatacgttgtttaataaaagtcgttattcaattacaattcatcgtgaatggcatct

SEQ ID NO: 50 - DNA, 21 bp, Primer
cccagatgcgaagttaagtgc

SEQ ID NO: 51 - DNA, 25 bp, Primer
attacgaaatggcctgtatgggtag

SEQ ID NO: 52 - DNA, 118 bp, Primer
tactcttgttcaatcagttagttatctttgttcaatagtgtggttggtaagcacacaccatagcttcaaaatgtttctactccttttttactcttccagacatggaggcccagaatac

SEQ ID NO: 53 - DNA, 97 bp, Primer
cccagatgcgaagttaagtgcgcagaaagtaatatcatgcgtcaatcgtatgtgaatgctggtcgctatactggcacacaccatagcttcaaaatgt

SEQ ID NO: 54 - DNA, 100 bp, Primer
attacgaaatggcctgtatgggtagattcttgttatgtttttacatacgttgtttaataaaagtcgttattcattacaattcatcgtgaatggcatcttc

SEQ ID NO: 55 - DNA, 20 bp, Primer
ttaccacggtgctccagttg

SEQ ID NO: 56 - DNA, 20 bp, Primer
aaccaagtcagcagcagaag

SEQ ID NO: 57 - DNA, 20 bp, Primer
tgcggcacagaagagtaacc

SEQ ID NO: 58 - DNA, 20 bp, Primer
ggcgataaacgataggcaac

SEQ ID NO: 59 - DNA, 22 bp, Primer
tccgctaagaacaactaagtga

SEQ ID NO: 60 - DNA, 22 bp, Primer
cactggctgtaaacggacctat

SEQ ID NO: 61 - DNA, 21 bp, Primer
tgcaaacccagtgtaagacgc

SEQ ID NO: 62 - DNA, 22 bp, Primer
atatggttcgagaacaggcatc

SEQ ID NO: 63 - DNA, 22 bp, Primer
agcacgacatagaagtgaaacc

SEQ ID NO: 64 - DNA, 22 bp, Primer
cgcaagggcaaacaggatagac

SEQ ID NO: 65 - DNA, 21 bp, Primer
cgattgagtcgaacaccctga

SEQ ID NO: 66 - DNA, 19 bp, Primer
cttgggtgcgtaggtctgg

SEQ ID NO: 67 - DNA, 22 bp, Primer
gtcttgtaaccaatggcgaaac

SEQ ID NO: 68 - DNA, 20 bp, Primer
gccaccacgattgacgaaca

SEQ ID NO: 69 - DNA, 22 bp, Primer
ttaacagcgacttgcccacagg

SEQ ID NO: 70 - DNA, 21 bp, Primer
agctagtctgtgacctgtacg

SEQ ID NO: 71 - DNA, 26 bp, Primer
tgcacgtgataatatgttaccctgtc

SEQ ID NO: 72 - DNA, 26 bp, Primer
ggaggaggatgagataagtagtttcc

SEQ ID NO: 73 - DNA, 22 bp, Primer
aaaactctggcggctaaactgg

SEQ ID NO: 74 - DNA, 25 bp, Primer
catcaatactggcgataagcgggac

SEQ ID NO: 75 - DNA, 27 bp, Primer
tccttggactctttattcgacttcatc

SEQ ID NO: 76 - DNA, 22 bp, Primer
cgcattataagtggtgtgccga

SEQ ID NO: 77 - DNA, 22 bp, Primer
atgctgtgcttgggtgttttga